European Patent Application EP 4 495 261 A1, published January 22, 2025. Title: DETECTION OF CORTICOSTEROID EFFICIENCY BY ANALYSING THE RS37973 AND RS28362491 POLYMORPHISMS. Applicant: UNIVERSITE DE VERSAILLES-SAINT-QUENTIN-EN-YVELINES. Application EP. The sequence listing filed with the application follows.

SEQUENCE LISTING (6 sequences)

SEQ ID NO: 1 - DNA, 1100 bp, Homo sapiens
  source 1..1100: mol_type = genomic DNA
gaaggtatccccagcctgtacctaatacagtgcccagcactaaagcagctcagatgccagtgaatggtggccactgggaggcctgtcagtgggtgccagtagcggtctcttcagagaaaaagaaaactcccctctgccagatcagtattttatgagctgtgaaccaaaaccattgctaccaccatcactataattctatccacagtaattatcataaaggcctaacaatgccttgtagatgaacattctgagtaactgctctataaccaggagatttaagaccgcaccaaaaaccagtagagggttatactttactgggcacaagtcgtttatgataacgaaattgtagtttaatctgtgaagagatgtgaatgtaactgagacacgcttaaatggaatatacagatgagctttatttttatatctggcatgcttggatccatgccgaccctccagctgctcgggcctgcccttaggggctatggaccgcatgactctatcagcggcactgccaccgccgccgcctccgtgctgcctgcgttccccgaccattgggcccggcaggcgcttcctgggggcttccctaccggctccagcccttgggattcgggagcgccctgctaggaagccagagccccgcaggggccgcggcgtccaggccgcctaacgcgcgcccctcgcccggcgccccgaagcggccccgaggggcgggagccgaggcgagcggcaaggccgggccgggggcgcacagcgcccctagaagtgcgggcttcccccacccccggcagcgaccctacctcccgcccccgctgcgtgcgcgcgtgtgtccgtctgtctgtatgctctctcgacgtcagtgggaatttccagccaggaagtgagagagtgagcgagacagaaagagagagaagtgcaccagcgagccggggcaggaagaggaggtttcgccaccggagcggcccggcgacgcgctgacagcttcccctgcccttcccgtcggtcgggccgccagccgccgcagccctcggcctgcacgcagccaccggccccgctcccggagcccagcgccgccgaggccgcagccgcccggccagtaaggc

SEQ ID NO: 2 - DNA, 1100 bp, Homo sapiens
  source 1..1100: mol_type = genomic DNA
ctagtatgctttctcgtctgaacacacaaggaagaaaagaaggatggctcctgtacgtgaaagtgacccctgcatatagtgcctgaaatcagaggaagcttgtcagtgtgggcagacaccacgagcagaccaatttgacattgtgcttctcttttaacctcttgaaaattaatgaaagttatctgatgaagatccttacattaattgctcccgattaaggtttaaaaccttggtttactgtggggtaaatttatgtttttgatagtcatccaaaatctttgtacgctttcagtttcattacagaataaaaaacaaatttaccacaatggattattacattacatctggtatttattcctcccaagaagctatctgcttcggaaaagccaggggcgcccttcattaatatatctaactgatggtgtaatgacataaaattccttgttgacccctgctattcagtgttattgtcttggaacatagaacttgataatctcttttcactgcataactacaaatgttaggctgtaagagtattttactttgttcatgcaggttccagacatttctcctgatcaccagaagttcttttgattaataaggctactggtcacgaaaactcagcttactaaaagagatccagtcttctggttctaactaaaacatcccaccggatgcaggtgtacttgcaaattaaagtttgcctcatgtgtcctgtgtctcaagtcatacagacggcccaggagggtggagcccctgcaacctgcctagcggggcgtttgcgtgtctgggggtgtcgggacacgcgcaggacacacacagtcccactttcctagtctcgcacttacctcaaggctgtcaacttttacgctcctccctgcgcgcacagcccccacctcacgctgccacccctcacgccccgccttcaaagtaggaggcaccattgtcattggacactgcttctctcactcctattccagaaccaatcactcgagttctagtggggagcgcctaagccaatggaaatgctcgctgcggcagctgccgggtcctgggcgctgggaggcggtgccgggggcggggtgcggctggggcgaatt

SEQ ID NO: 3 - DNA, 18 bp, synthetic construct
  source 1..18: mol_type = other DNA
ttggatccatgccgaccc

SEQ ID NO: 4 - DNA, 20 bp, synthetic construct
  source 1..20: mol_type = other DNA
tcactctctcacttcctggc

SEQ ID NO: 5 - DNA, 23 bp, synthetic construct
  source 1..23: mol_type = other DNA
acataaaattccttgttgacccc

SEQ ID NO: 6 - DNA, 23 bp, synthetic construct
  source 1..23: mol_type = other DNA
cggtgggatgttttagttagaac